European Patent Application EP 4 806 458 A1, published September 16, 2026. Title: 用于降糖的酰化胰岛素. Applicant: 甘李药业股份有限公司. The sequence listing filed with the application follows.

SEQUENCE LISTING (2 sequences)

SEQ ID NO: 1 - protein, 21 aa, artificial sequence
GIVEQCCTSICSLEQLENYCN

SEQ ID NO: 2 - protein, 29 aa, artificial sequence
FVNQHLCGSHLVEALHLVCGERGFHYTPK